European Patent Application EP 4 410 770 A1, published August 7, 2024. Title: PRODUCTION METHOD FOR PURIFIED DICHLOROACETIC ACID. Applicant: Sumitomo Chemical Company, Limited. Application EP 22876216.7, filed September 27, 2022. The sequence listing filed with the application follows.

SEQUENCE LISTING (12 sequences)

SEQ ID NO: 1 - RNA, 21 nt, synthetic construct
  misc_feature 1..21: note = Synthetic oligonucleotide
  modified_base 7: mod_base = um
  modified_base 17: mod_base = um
  modified_base 20..21: mod_base = OTHER; note = dT
  source 1..21: mol_type = other RNA
atggaanactcttggtnacnn

SEQ ID NO: 2 - RNA, 21 nt, synthetic construct
  misc_feature 1..21: note = Synthetic oligonucleotide
  modified_base 2: mod_base = um
  modified_base 12: mod_base = um
  modified_base 14..15: mod_base = um
  modified_base 19: mod_base = um
  modified_base 5..6: mod_base = cm
  modified_base 16..17: mod_base = cm
  modified_base 20..21: mod_base = OTHER; note = dT
  source 1..21: mol_type = other RNA
gnaannaagagnannnnannn

SEQ ID NO: 3 - RNA, 36 nt, synthetic construct
  misc_feature 1..36: note = Synthetic oligonucleotide
  source 1..36: mol_type = other RNA
agagccagccttcttattgttttagagctatgctgt

SEQ ID NO: 4 - RNA, 23 nt, synthetic construct
  misc_feature 1..23: note = Synthetic oligonucleotide
  source 1..23: mol_type = other RNA
ccatgagaagtatgacaacagcc

SEQ ID NO: 5 - RNA, 25 nt, synthetic construct
  misc_feature 1..25: note = Synthetic oligonucleotide
  source 1..25: mol_type = other RNA
ggctgttgtcatacttctcatggtt

SEQ ID NO: 6 - RNA, 67 nt, synthetic construct
  misc_feature 1..67: note = Synthetic oligonucleotide
  source 1..67: mol_type = other RNA
acagcatagcaagttaaaataaggctagtccgttatcaacttgaaaaagtggcaccgagtcggtgct

SEQ ID NO: 7 - RNA, 94 nt, synthetic construct
  misc_feature 1..94: note = Synthetic oligonucleotide
  source 1..94: mol_type = other RNA
gttttcccttttcaaagaaatctcctgggcacctatcttcttaggtgccctcccttgtttaaacctgaccagttaaccggctggttaggttttt

SEQ ID NO: 8 - RNA, 100 nt, synthetic construct
  misc_feature 1..100: note = Synthetic oligonucleotide
  source 1..100: mol_type = other RNA
agtcctcatctccctcaagcgttttagagctagtaatagcaagttaaaataaggctagtccgttatcaacttgaaaaagtggcaccgagtcggtgctttt

SEQ ID NO: 9 - RNA, 113 nt, synthetic construct
  misc_feature 1..113: note = Synthetic oligonucleotide
  source 1..113: mol_type = other RNA
gcagatgtagtgtttccacagtttaagagctatgctggaaacagcatagcaagtttaaataaggctagtccgttatcaacttgaaaaagtggcaccgagtcggtgcttttttt

SEQ ID NO: 10 - RNA, 113 nt, synthetic construct
  misc_feature 1..113: note = Synthetic oligonucleotide
  modified_base 1: mod_base = OTHER; note = dA
  modified_base 8: mod_base = OTHER; note = dA
  modified_base 17..18: mod_base = OTHER; note = dA
  modified_base 2: mod_base = OTHER; note = dG
  modified_base 19: mod_base = OTHER; note = dG
  modified_base 3: mod_base = OTHER; note = dT
  modified_base 6: mod_base = OTHER; note = dT
  modified_base 9: mod_base = OTHER; note = dT
  modified_base 11: mod_base = OTHER; note = dT
  modified_base 15: mod_base = OTHER; note = dT
  modified_base 4..5: mod_base = OTHER; note = dC
  modified_base 7: mod_base = OTHER; note = dC
  modified_base 10: mod_base = OTHER; note = dC
  modified_base 12..14: mod_base = OTHER; note = dC
  modified_base 16: mod_base = OTHER; note = dC
  modified_base 20: mod_base = OTHER; note = dC
  source 1..113: mol_type = other RNA
nnnnnnnnnnnnnnnnnnnngtttaagagctatgctggtaacagcatagcaagtttaaataaggctagtccgttatcaacttgaaaaagtggcaccgagtcggtgcttttttt

SEQ ID NO: 11 - RNA, 113 nt, synthetic construct
  misc_feature 1..113: note = Synthetic oligonucleotide
  modified_base 1: mod_base = OTHER; note = am
  modified_base 2: mod_base = gm
  modified_base 3: mod_base = um
  modified_base 110..112: mod_base = um
  source 1..113: mol_type = other RNA
nnncctcatctccctcaagcgtttaagagctatgctggtaacagcatagcaagtttaaataaggctagtccgttatcaacttgaaaaagtggcaccgagtcggtgctttnnnt

SEQ ID NO: 12 - RNA, 50 nt, synthetic construct
  misc_feature 1..50: note = Synthetic oligonucleotide
  source 1..50: mol_type = other RNA
aaggctagtccgttatcaacttgaaaaagtggcaccgagtcggtgctttt